European Patent Specification EP 3 565 844 B1, published March 1, 2023. Title: METHODS OF TREATING CANCER WITH ANTI-PD-1 ANTIBODIES. Applicant: Tesaro, Inc. The sequence listing filed with the application follows.

SEQUENCE LISTING (14 sequences)

SEQ ID NO: 1 - protein, 117 aa, Artificial Sequence
  Synthetic Polypeptide
EVQLLESGGGLVQPGGSLRLSCAASGFTFSSYDMSWVRQAPGKGLEWVSTISGGGSYTYYQDSVKGRFTISRDNSKNTLYLQMNSLRAEDTAVYYCASPYYAMDYWGQGTTVTVSSA

SEQ ID NO: 2 - protein, 108 aa, Artificial Sequence
  Synthetic Polypeptide
DIQLTQSPSFLSAYVGDRVTITCKASQDVGTAVAWYQQKPGKAPKLLIYWASTLHTGVPSRFSGSGSGTEFTLTISSLQPEDFATYYCQHYSSYPWTFGQGTKLEIKR

SEQ ID NO: 3 - protein, 443 aa, Artificial Sequence
  Synthetic Polypeptide
EVQLLESGGGLVQPGGSLRLSCAASGFTFSSYDMSWVRQAPGKGLEWVSTISGGGSYTYYQDSVKGRFTISRDNSKNTLYLQMNSLRAEDTAVYYCASPYYAMDYWGQGTTVTVSSASTKGPSVFPLAPCSRSTSESTAALGCLVKDYFPEPVTVSWNSGALTSGVHTFPAVLQSSGLYSLSSVVTVPSSSLGTKTYTCNVDHKPSNTKVDKRVESKYGPPCPPCPAPEFLGGPSVFLFPPKPKDTLMISRTPEVTCVVVDVSQEDPEVQFNWYVDGVEVHNAKTKPREEQFNSTYRVVSVLTVLHQDWLNGKEYKCKVSNKGLPSSIEKTISKAKGQPREPQVYTLPPSQEEMTKNQVSLTCLVKGFYPSDIAVEWESNGQPENNYKTTPPVLDSDGSFFLYSRLTVDKSRWQEGNVFSCSVMHEALHNHYTQKSLSLSLGK

SEQ ID NO: 4 - protein, 214 aa, Artificial Sequence
  Synthetic Polypeptide
DIQLTQSPSFLSAYVGDRVTITCKASQDVGTAVAWYQQKPGKAPKLLIYWASTLHTGVPSRFSGSGSGTEFTLTISSLQPEDFATYYCQHYSSYPWTFGQGTKLEIKRTVAAPSVFIFPPSDEQLKSGTASVVCLLNNFYPREAKVQWKVDNALQSGNSQESVTEQDSKDSTYSLSSTLTLSKADYEKHKVYACEVTHQGLSSPVTKSFNRGEC

SEQ ID NO: 5 - DNA, 1329 bp, Artificial Sequence
  Synthetic Polynucleotide
gaggtgcagctgttggagtctgggggaggcttggtacagcctggggggtccctgagactctcctgtgcagcctctggattcactttcagtagctatgacatgtcttgggtccgccaggctccagggaaggggctggagtgggtctcaaccattagtggtggtggtagttacacctactatcaagacagtgtgaaggggcggttcaccatctccagagacaattccaagaacacgctgtatctgcaaatgaacagcctgagagccgaggacacggccgtatattactgtgcgtccccttactatgctatggactactgggggcaagggaccacggtcaccgtctcctcagcatccaccaagggcccatcggtcttcccgctagcaccctgctccaggagcacctccgagagcacagccgccctgggctgcctggtcaaggactacttccccgaaccagtgacggtgtcgtggaactcaggcgccctgaccagcggcgtgcacaccttcccggctgtcctacagtcctcaggactctactccctcagcagcgtggtgaccgtgccctccagcagcttgggcacgaagacctacacctgcaacgtagatcacaagcccagcaacaccaaggtggacaagagagttgagtccaaatatggtcccccatgcccaccatgcccagcacctgagttcctggggggaccatcagtcttcctgttccccccaaaacccaaggacactctcatgatctcccggacccctgaggtcacgtgcgtggtggtggacgtgagccaggaagaccccgaggtccagttcaactggtacgtggatggcgtggaggtgcataatgccaagacaaagccgcgggaggagcagttcaacagcacgtaccgtgtggtcagcgtcctcaccgtcctgcaccaggactggctgaacggcaaggagtacaagtgcaaggtctccaacaaaggcctcccgtcctccatcgagaaaaccatctccaaagccaaagggcagccccgagagccacaggtgtacaccctgcccccatcccaggaggagatgaccaagaaccaggtcagcctgacctgcctggtcaaaggcttctaccccagcgacatcgccgtggagtgggagagcaatgggcagccggagaacaactacaagaccacgcctcccgtgctggactccgacggctccttcttcctctacagcaggctaaccgtggacaagagcaggtggcaggaggggaatgtcttctcatgctccgtgatgcatgaggctctgcacaaccactacacacagaagagcctctccctgtctctgggtaaa

SEQ ID NO: 6 - DNA, 642 bp, Artificial Sequence
  Synthetic Polynucleotide
gacatccagttgacccagtctccatccttcctgtctgcatatgtaggagacagagtcaccatcacttgcaaggccagtcaggatgtgggtactgctgtagcctggtatcagcaaaaaccagggaaagcccctaagctcctgatctattgggcatccaccctgcacactggggtcccatcaaggttcagcggcagtggatctgggacagaattcactctcacaatcagcagcctgcagcctgaagattttgcaacttattactgtcagcattatagcagctatccgtggacgtttggccaggggaccaagctggagatcaaacggactgtggctgcaccatctgtcttcatcttcccgccatctgatgagcaattgaaatctggaactgcctctgttgtgtgcctgctgaataacttctatcccagagaggccaaagtacagtggaaggtggataacgccctccaatcgggtaactcccaggagagtgtcacagagcaggacagcaaggacagcacctacagcctcagcagcaccctgacgctgagcaaagcagactacgagaaacacaaagtctacgcctgcgaagtcacccatcagggcctcagctcgcccgtcacaaagagcttcaacaggggagagtgt

SEQ ID NO: 7 - protein, 116 aa, Artificial Sequence
  Synthetic Polypeptide
EVQLLESGGGLVQPGGSLRLSCAASGFTFSSYDMSWVRQAPGKGLEWVSTISGGGSYTYYQDSVKGRFTISRDNSKNTLYLQMNSLRAEDTAVYYCASPYYAMDYWGQGTTVTVSS

SEQ ID NO: 8 - protein, 107 aa, Artificial Sequence
  Synthetic Polypeptide
DIQLTQSPSFLSAYVGDRVTITCKASQDVGTAVAWYQQKPGKAPKLLIYWASTLHTGVPSRFSGSGSGTEFTLTISSLQPEDFATYYCQHYSSYPWTFGQGTKLEIK

SEQ ID NO: 9 - protein, 5 aa, Artificial Sequence
  Synthetic Oligopeptide
SYDMS

SEQ ID NO: 10 - protein, 17 aa, Artificial Sequence
  Synthetic Oligopeptide
TISGGGSYTYYQDSVKG

SEQ ID NO: 11 - protein, 7 aa, Artificial Sequence
  Synthetic Oligopeptide
PYYAMDY

SEQ ID NO: 12 - protein, 11 aa, Artificial Sequence
  Synthetic Oligopeptide
KASQDVGTAVA

SEQ ID NO: 13 - protein, 7 aa, Artificial Sequence
  Synthetic Oligopeptide
WASTLHT

SEQ ID NO: 14 - protein, 9 aa, Artificial Sequence
  Synthetic Oligopeptide
QHYSSYPWT